European Patent Specification EP 3 904 387 B1, published February 11, 2026. Title: MONOCLONAL ANTIBODIES THAT BIND SPECIFICALLY TO HUMAN TRBV9. Applicant: JSC "BIOCAD". Application PCT/RU2019/050257. The sequence listing filed with the application follows.

SEQUENCE LISTING (22 sequences)

SEQ ID NO: 1 - protein, 5 aa, Artificial
  The HCDR1 sequence of the parental antibody TRBV9-2
DYLVH

SEQ ID NO: 2 - protein, 17 aa, Artificial
  The HCDR2 sequence of the parental antibody TRBV9-2
WINTYTGTPTYADDFEG

SEQ ID NO: 3 - protein, 13 aa, Artificial
  The HCDR3 sequence of the parental antibody TRBV9-2
SWRRGLRGIGFDY

SEQ ID NO: 4 - protein, 11 aa, Artificial
  The LCDR1 sequence of the parental antibody TRBV9-2
KASKSINKYLA

SEQ ID NO: 5 - protein, 7 aa, Artificial
  The LCDR2 sequence of the parental antibody TRBV9-2
DGSTLQS

SEQ ID NO: 6 - protein, 9 aa, Artificial
  The LCDR3 sequence of the parental antibody TRBV9-2
QQHNEYPPT

SEQ ID NO: 7 - DNA, 366 bp, Artificial
  The nucleotide sequence of the variable domain of the heavy chain of the parental antibody TRBV9-2
caaatacaactggtgcagagcgggccagaattgagagaacccggagaatctgtgaagctgagttgtaaggccagcggatacactttcactgactatctcgtgcactgggtgaaacaggctcccggtaagggattgaaatggatgggatggatcaatacttataccggcacacctacatatgcagacgatttcgaggggcgatttgtgttcagtttggaggcctctgccagcacggcgaacctgcagatatcgaatctcaagaatgaggacaccgccacgtatttctgcgctagatcttggagacgcggattgagaggtatcggattcgactactggggacaaggcgtcttcgtgactgtatcatcc

SEQ ID NO: 8 - protein, 122 aa, Artificial
  The amino acid sequence of the variable domain of the heavy chain of the parental antibody TRBV9-2
QIQLVQSGPELREPGESVKLSCKASGYTFTDYLVHWVKQAPGKGLKWMGWINTYTGTPTYADDFEGRFVFSLEASASTANLQISNLKNEDTATYFCARSWRRGLRGIGFDYWGQGVFVTVSS

SEQ ID NO: 9 - DNA, 321 bp, Artificial
  The nucleotide sequence of the light chain variable domain of the parental antibody TRBV9-2
gatgtacagatgacacaatcaccctacaaccttgctgcttcccctggggaaagtgtcagtatcaattgcaaggcatcgaagtcgatcaacaagtatcttgcgtggtatcagcagaagccaggaaagcccaacaagctcctgatctatgacggctctacactgcaatctggcataccttcgcggttttctggctcggggtccgggactgacttcactcttacaatacgaggacttgaacccgaagacttcggcctgtattactgccagcagcacaatgagtatccacctaccttcggggctggcaccaagttggagcttaag

SEQ ID NO: 10 - protein, 107 aa, Artificial
  The amino acid sequence of the light chain variable domain of the parent antibody TRBV9-2
DVQMTQSPYNLAASPGESVSINCKASKSINKYLAWYQQKPGKPNKLLIYDGSTLQSGIPSRFSGSGSGTDFTLTIRGLEPEDFGLYYCQQHNEYPPTFGAGTKLELK

SEQ ID NO: 11 - DNA, 639 bp, Artificial
  The nucleotide sequence of the light chain of the parental antibody TRBV9-2
gacgtgcagatgacccagtccccctacaacctggccgcctcccccggcgagtccgtgtccatcaactgcaaggcctccaagtccatcaacaagtacctggcctggtaccagcagaagcccggcaagcccaacaagctgctgatctacgacggctccaccctgcagtccggcatcccctccaggttctccggctccggctccggcaccgacttcaccctgaccatcaggggcctggagcccgaggacttcggcctgtactactgccagcagcacaacgagtacccccccaccttcggcgccggcaccaagctggagctgaagcgaactgtggctgcaccatctgtcttcatcttcccgccatctgatgagcagttgaaatctggaactgcctctgtcgtgtgcctgctgaataacttctatcccagagaggccaaagtacagtggaaggtggataacgccctccaatcgggtaactcccaggagagtgtcacagagcaggacagcaaggacagcacctacagcctcagcagcaccctgacgctgagcaaagcagactacgagaaacacaaagtctacgcctgcgaagtcacccatcagggcctgtcctcgcccgtcacaaagagcttcaacaggggagag

SEQ ID NO: 12 - protein, 213 aa, Artificial
  The amino acid sequence of the light chain of the parental antibody TRBV9-2
DVQMTQSPYNLAASPGESVSINCKASKSINKYLAWYQQKPGKPNKLLIYDGSTLQSGIPSRFSGSGSGTDFTLTIRGLEPEDFGLYYCQQHNEYPPTFGAGTKLELKRTVAAPSVFIFPPSDEQLKSGTASVVCLLNNFYPREAKVQWKVDNALQSGNSQESVTEQDSKDSTYSLSSTLTLSKADYEKHKVYACEVTHQGLSSPVTKSFNRGE

SEQ ID NO: 13 - DNA, 1365 bp, Artificial
  The nucleotide sequence of the heavy chain of the parental antibody TRBV9-2
cagatccagctggtgcagtccggccccgagctgagggagcccggcgagtccgtgaagctgtcctgcaaggcctccggctacaccttcaccgactacctggtgcactgggtgaagcaggcccccggcaagggcctgaagtggatgggctggatcaacacctacaccggcacccccacctacgccgacgacttcgagggcaggttcgtgttctccctggaggcctccgcctccaccgccaacctgcagatctccaacctgaagaacgaggacaccgccacctacttctgcgccaggtcctggaggaggggcctgaggggcatcggcttcgactactggggccagggcgtgttcgtgaccgtgtcctccgcctccaccaagggcccatcggtcttccccctggcaccctcctccaagagcacctctgggggcacagcggccctgggctgcctggtcaaggactacttccccgaaccggtgacggtgtcgtggaactcaggcgccctgaccagcggcgtgcacaccttcccggctgtcctacagtcctcaggactctactccctcagcagcgtggtgactgtgccctctagcagcttgggcacccagacctacatctgcaacgtgaatcacaagcccagcaacaccaaggtggacaagaaagttgagcccccgaaatcttgtgacaaaactcacacatgcccaccgtgcccagcacctgaactcctggggggaccgtcagtcttcctcttccccccaaaacccaaggacaccctcatgatctcccggacccctgaggtcacatgcgtggtggtggacgtgagccacgaagaccctgaggtcaagttcaactggtacgtggacggcgtggaggtgcataatgccaagacaaagccgcgggaggagcagtacaacagcacgtaccgtgtggtcagcgtcctcaccgtcctgcaccaggactggctgaatggcaaggagtacaagtgcaaggtctccaacaaagccctcccagcccccatcgagaaaaccatctccaaagccaaagggcagccccgagaaccacaggtgtacaccctgcccccatcccgggatgagctgaccaagaaccaggtcagcctgacctgcctggtcaaaggcttctatcccagcgacatcgccgtggagtgggagagcaatgggcagccggagaacaactacaagaccacgcctcccgtgctggactccgacggctccttcttcctctacagcaagctcaccgtggacaagagcaggtggcagcaggggaacgtcttctcatgctccgtgatgcatgaggctctgcacaaccactacacgcagaagagcctctccctgtctccgggtaaatgataa

SEQ ID NO: 14 - protein, 453 aa, Artificial
  The amino acid sequence of heavy chain of the parental antibody TRBV9-2
QIQLVQSGPELREPGESVKLSCKASGYTFTDYLVHWVKQAPGKGLKWMGWINTYTGTPTYADDFEGRFVFSLEASASTANLQISNLKNEDTATYFCARSWRRGLRGIGFDYWGQGVFVTVSSASTKGPSVFPLAPSSKSTSGGTAALGCLVKDYFPEPVTVSWNSGALTSGVHTFPAVLQSSGLYSLSSVVTVPSSSLGTQTYICNVNHKPSNTKVDKKVEPPKSCDKTHTCPPCPAPELLGGPSVFLFPPKPKDTLMISRTPEVTCVVVDVSHEDPEVKFNWYVDGVEVHNAKTKPREEQYNSTYRVVSVLTVLHQDWLNGKEYKCKVSNKALPAPIEKTISKAKGQPREPQVYTLPPSRDELTKNQVSLTCLVKGFYPSDIAVEWESNGQPENNYKTTPPVLDSDGSFFLYSKLTVDKSRWQQGNVFSCSVMHEALHNHYTQKSLSLSPGK

SEQ ID NO: 15 - DNA, 366 bp, Artificial
  The nucleotide sequence of the variable heavy chain of the antibody MA-042
caggtgcaacttgttcagtcggggagcgaacttaagaagccaggggaaagtgtaaaagtgagctgcaaagcctcaggctacacgtttaccgattatcttgtgcattgggttagacaggctccaggtcaaggactggaatggatgggatggatcaatacctatacagggacacccacatatgccgatgactttgagggacggtttgtcttctcacttgataccagtgtttccactgctaacctccagataagcagcctgaaggcagaggacaccgccgtttatttctgcgcccgatcatggaggagaggcttgcgaggaattggattcgattactggggtcagggcactttagtcactgtctctagc

SEQ ID NO: 16 - protein, 122 aa, Artificial
  The amino acid sequence of the variable domain of the heavy chain of the parental antibody MA-042
QVQLVQSGSELKKPGESVKVSCKASGYTFTDYLVHWVRQAPGQGLEWMGWINTYTGTPTYADDFEGRFVFSLDTSVSTANLQISSLKAEDTAVYFCARSWRRGLRGIGFDYWGQGTLVTVSS

SEQ ID NO: 17 - DNA, 321 bp, Artificial
  The nucleotide sequence of the variable light chain of the antibody MA-042
gacatacagatgactcaaagcccttattcgctcagtgcgtcggtcggggacagagtaaccatcacctgcaaggcgtcaaagtcaatcaataagtatctggcgtggttccagcagaagccaggaaagcctaacaagctattaatatacgatgggtctaccctccaatccggggtcccttcacgattttctggaagcggctcaggaaccgatttcacgctgaccatcagtagcttggagcctgaggactttgccacttattattgccagcagcacaacgagtatcctcccaccttcggacagggtacaaaactggagatcaag

SEQ ID NO: 18 - protein, 107 aa, Artificial
  The amino acid sequence of variable light chain of the antibody MA-042
DIQMTQSPYSLSASVGDRVTITCKASKSINKYLAWFQQKPGKPNKLLIYDGSTLQSGVPSRFSGSGSGTDFTLTISSLEPEDFATYYCQQHNEYPPTFGQGTKLEIK

SEQ ID NO: 19 - DNA, 1356 bp, Artificial
  The nucleotide sequence of the heavy chain of the antibody MA-042
caggtgcaacttgttcagtcggggagcgaacttaagaagccaggggaaagtgtaaaagtgagctgcaaagcctcaggctacacgtttaccgattatcttgtgcattgggttagacaggctccaggtcaaggactggaatggatgggatggatcaatacctatacagggacacccacatatgccgatgactttgagggacggtttgtcttctcacttgataccagtgtttccactgctaacctccagataagcagcctgaaggcagaggacaccgccgtttatttctgcgcccgatcatggaggagaggcctacgaggaatcggattcgattactggggtcagggcactttagtcactgtctctagcgctagcaccaagggcccatcggtcttccccctggcaccctcctccaagagcacctctgggggcacagcggccctgggctgcctggtcaaggactacttccccgaaccggtgacggtgtcgtggaactcaggcgccctgaccagcggcgtgcacaccttcccggctgtcctacagtcctcaggactctactccctcagcagcgtggtgaccgtgccctccagcagcttgggcacccagacctacatctgcaacgtgaatcacaagcccagcaacaccaaggtggacaagagagttgagcccaaatcttgtgacaaaactcacacatgcccaccgtgcccagcacctgaactcctggggggaccgtcagtcttcctcttccccccaaaacccaaggacaccctcatgatctcccggacccctgaggtcacatgcgtggtggtggacgtgagccacgaagaccctgaggtcaagttcaactggtacgtggacggcgtggaggtgcataatgccaagacaaagccgcgggaggagcagtacaacagcacgtaccgtgtggtcagcgtcctcaccgtcctgcaccaggactggctgaatggcaaggagtacaagtgcaaggtctccaacaaagccctcccagcccccatcgagaaaaccatctccaaagccaaagggcagccccgagaaccacaggtgtacaccctgcccccatcccgggaggagatgaccaagaaccaggtcagcctgacctgcctggtcaaaggcttctatcccagcgacatcgccgtggagtgggagagcaatgggcagccggagaacaactacaagaccacgcctcccgtgctggactccgacggctccttcttcctctatagcaagctcaccgtggacaagagcaggtggcagcaggggaacgtcttctcatgctccgtgatgcatgaggctctgcacaaccactacacgcagaaaagcctctccctgtccccgggtaaa

SEQ ID NO: 20 - protein, 452 aa, Artificial
  The amino acid sequence of the heavy chain of the antibody MA-042
QVQLVQSGSELKKPGESVKVSCKASGYTFTDYLVHWVRQAPGQGLEWMGWINTYTGTPTYADDFEGRFVFSLDTSVSTANLQISSLKAEDTAVYFCARSWRRGLRGIGFDYWGQGTLVTVSSASTKGPSVFPLAPSSKSTSGGTAALGCLVKDYFPEPVTVSWNSGALTSGVHTFPAVLQSSGLYSLSSVVTVPSSSLGTQTYICNVNHKPSNTKVDKRVEPKSCDKTHTCPPCPAPELLGGPSVFLFPPKPKDTLMISRTPEVTCVVVDVSHEDPEVKFNWYVDGVEVHNAKTKPREEQYNSTYRVVSVLTVLHQDWLNGKEYKCKVSNKALPAPIEKTISKAKGQPREPQVYTLPPSREEMTKNQVSLTCLVKGFYPSDIAVEWESNGQPENNYKTTPPVLDSDGSFFLYSKLTVDKSRWQQGNVFSCSVMHEALHNHYTQKSLSLSPGK

SEQ ID NO: 21 - DNA, 642 bp, Artificial
  The nucleotide sequence of the light chain of the antibody MA-042
gacatacagatgactcaaagcccttattcgctcagtgcgtcggtcggggacagagtaaccatcacctgcaaggcgtcaaagtcaatcaataagtatctggcgtggttccagcagaagccaggaaagcctaacaagctattaatatacgatgggtctaccctccaatccggggtcccttcacgattttctggaagcggctcaggaaccgatttcacgctgaccatcagtagcttggagcctgaggactttgccacttattattgccagcagcacaacgagtatcctcccaccttcggacagggtacaaaactggagatcaagcgtacggtggctgcaccatctgtcttcatcttcccgccatctgatgagcagttgaaatctggaactgcctctgttgtgtgcctgctgaataacttctatcccagagaggccaaagtacagtggaaggtggataacgccctccaatcgggtaactcccaggagagtgtcacagagcaggacagcaaggacagcacctacagcctcagcagcaccctgacgctgagcaaagcagactacgagaaacacaaagtctacgcctgcgaagtcacccatcagggcctgagctcgcccgtcacaaagagcttcaacaggggagagtgt

SEQ ID NO: 22 - protein, 214 aa, Artificial
  The amino acid sequence of a light chain of the antibody MA-042
DIQMTQSPYSLSASVGDRVTITCKASKSINKYLAWFQQKPGKPNKLLIYDGSTLQSGVPSRFSGSGSGTDFTLTISSLEPEDFATYYCQQHNEYPPTFGQGTKLEIKRTVAAPSVFIFPPSDEQLKSGTASVVCLLNNFYPREAKVQWKVDNALQSGNSQESVTEQDSKDSTYSLSSTLTLSKADYEKHKVYACEVTHQGLSSPVTKSFNRGEC